European Patent Specification EP 3 972 987 B1, published June 7, 2023. Title: ANTIGEN SPECIFIC IMMUNOTHERAPY FOR COVID-19 FUSION PROTEINS AND METHODS OF USE. Applicant: Akston Biosciences Corporation. The sequence listing filed with the application follows.

SEQUENCE LISTING (33 sequences)

SEQ ID NO: 1 - protein, 1273 aa, SARS-CoV-2 Surface Glycoprotein
MFVFLVLLPLVSSQCVNLTTRTQLPPAYTNSFTRGVYYPDKVFRSSVLHSTQDLFLPFFSNVTWFHAIHVSGTNGTKRFDNPVLPFNDGVYFASTEKSNIIRGWIFGTTLDSKTQSLLIVNNATNVVIKVCEFQFCNDPFLGVYYHKNNKSWMESEFRVYSSANNCTFEYVSQPFLMDLEGKQGNFKNLREFVFKNIDGYFKIYSKHTPINLVRDLPQGFSALEPLVDLPIGINITRFQTLLALHRSYLTPGDSSSGWTAGAAAYYVGYLQPRTFLLKYNENGTITDAVDCALDPLSETKCTLKSFTVEKGIYQTSNFRVQPTESIVRFPNITNLCPFGEVFNATRFASVYAWNRKRISNCVADYSVLYNSASFSTFKCYGVSPTKLNDLCFTNVYADSFVIRGDEVRQIAPGQTGKIADYNYKLPDDFTGCVIAWNSNNLDSKVGGNYNYLYRLFRKSNLKPFERDISTEIYQAGSTPCNGVEGFNCYFPLQSYGFQPTNGVGYQPYRVVVLSFELLHAPATVCGPKKSTNLVKNKCVNFNFNGLTGTGVLTESNKKFLPFQQFGRDIADTTDAVRDPQTLEILDITPCSFGGVSVITPGTNTSNQVAVLYQDVNCTEVPVAIHADQLTPTWRVYSTGSNVFQTRAGCLIGAEHVNNSYECDIPIGAGICASYQTQTNSPRRARSVASQSIIAYTMSLGAENSVAYSNNSIAIPTNFTISVTTEILPVSMTKTSVDCTMYICGDSTECSNLLLQYGSFCTQLNRALTGIAVEQDKNTQEVFAQVKQIYKTPPIKDFGGFNFSQILPDPSKPSKRSFIEDLLFNKVTLADAGFIKQYGDCLGDIAARDLICAQKFNGLTVLPPLLTDEMIAQYTSALLAGTITSGWTFGAGAALQIPFAMQMAYRFNGIGVTQNVLYENQKLIANQFNSAIGKIQDSLSSTASALGKLQDVVNQNAQALNTLVKQLSSNFGAISSVLNDILSRLDKVEAEVQIDRLITGRLQSLQTYVTQQLIRAAEIRASANLAATKMSECVLGQSKRVDFCGKGYHLMSFPQSAPHGVVFLHVTYVPAQEKNFTTAPAICHDGKAHFPREGVFVSNGTHWFVTQRNFYEPQIITTDNTFVSGNCDVVIGIVNNTVYDPLQPELDSFKEELDKYFKNHTSPDVDLGDISGINASVVNIQKEIDRLNEVAKNLNESLIDLQELGKYEQYIKWPWYIWLGFIAGLIAIVMVTIMLCCMTSCCSCLKGCCSCGSCCKFDEDDSEPVLKGVKLHYT

SEQ ID NO: 2 - protein, 254 aa, SARS-Cov-2 RBD
PNITNLCPFGEVFNATRFASVYAWNRKRISNCVADYSVLYNSASFSTFKCYGVSPTKLNDLCFTNVYADSFVIRGDEVRQIAPGQTGKIADYNYKLPDDFTGCVIAWNSNNLDSKVGGNYNYLYRLFRKSNLKPFERDISTEIYQAGSTPCNGVEGFNCYFPLQSYGFQPTNGVGYQPYRVVVLSFELLHAPATVCGPKKSTNLVKNKCVNFNFNGLTGTGVLTESNKKFLPFQQFGRDIADTTDAVRDPQTLE

SEQ ID NO: 3 - protein, 7 aa, Artificial Sequence
  Synthetic Linker
GGGSGGG

SEQ ID NO: 4 - protein, 21 aa, Artificial Sequence
  Synthetic Linker
GGGGGQGGGGQGGGGQGGGGG

SEQ ID NO: 5 - protein, 8 aa, Artificial Sequence
  Synthetic Linker
GGGSGGGS

SEQ ID NO: 6 - protein, 226 aa, Artificial Sequence
  Synthetic Fc Fragment
DKTHTCPPCPAPELLGGPSVFLFPPKPKDTLMISRTPEVTCVVVDVSHEDPEVKFNWYVDGVEVHNAKTKPREEQYNSTYRVVSVLTVLHQDWLNGKEYKCKVSNKALPAPIEKTISKAKGQPREPQVYTLPPSRDELTKNQVSLTCLVKGFYPSDIAVEWESNGQPENNYKTTPPVLDSDGSFFLYSKLTVDKSRWQQGNVFSCSVMHEALHNHYTQKSLSLSPG

SEQ ID NO: 7 - protein, 231 aa, Artificial Sequence
  Synthetic Fc Fragment
PKSSDKTHTCPPCPAPELLGGPSVFLFPPKPKDTLMISRTPEVTCVVVDVSHEDPEVKFNWYVDGVEVHNAKTKPREEQYNSTYRVVSVLTVLHQDWLNGKEYKCKVSNKALPAPIEKTISKAKGQPREPQVYTLPPSRDELTKNQVSLTCLVKGFYPSDIAVEWESNGQPENNYKTTPPVLDSDGSFFLYSKLTVDKSRWQQGNVFSCSVMHEALHNHYTQKSLSLSPGK

SEQ ID NO: 8 - protein, 194 aa, Artificial Sequence
  Synthetic SARS-Cov-2 RBD Analog
NITNLCPFGEVFNATRFASVYAWNRKRISNCVADYSVLYNSASFSTFKCYGVSPTKLNDLCFTNVYADSFVIRGDEVRQIAPGQTGKIADYNYKLPDDFTGCVIAWNSNNLDSKVGGNYNYLYRLFRKSNLKPFERDISTEIYQAGSTPCNGVEGFNCYFPLQSYGFQPTNGVGYQPYRVVVLSFELLHAPATV

SEQ ID NO: 9 - protein, 194 aa, Artificial Sequence
  Synthetic SARS-Cov-2 RBD Analog
QITNLCPFGEVFQATRFASVYAWNRKRISNCVADYSVLYNSASFSTFKCYGVSPTKLNDLMFTNVYADSFVIRGDEVRQIAPGQTGKIADYNYKLPDDFTGCVIAWNSNNLDSKVGGNYNYLYRLFRKSNLKPFERDISTEIYQAGSTPCNGVEGFNCYFPLQSYGFQPTNGVGYQPYRVVVLSFELLHAPATV

SEQ ID NO: 10 - protein, 92 aa, Artificial Sequence
  Synthetic SARS-Cov-2 RBD Analog
VIAWNSNNLDSKVGGNYNYLYRLFRKSNLKPFERDISTEIYQAGSTPCNGVEGFNCYFPLQSYGFQPTNGVGYQPYRVVVLSFELLHAPATV

SEQ ID NO: 11 - protein, 441 aa, Artificial Sequence
  Synthetic SARS-CoV-2-RBD-hIgG-Fc Fusion Protein
QITNLCPFGEVFQATRFASVYAWNRKRISNCVADYSVLYNSASFSTFKCYGVSPTKLNDLMFTNVYADSFVIRGDEVRQIAPGQTGKIADYNYKLPDDFTGCVIAWNSNNLDSKVGGNYNYLYRLFRKSNLKPFERDISTEIYQAGSTPCNGVEGFNCYFPLQSYGFQPTNGVGYQPYRVVVLSFELLHAPATVGGGGGQGGGGQGGGGQGGGGGDKTHTCPPCPAPELLGGPSVFLFPPKPKDTLMISRTPEVTCVVVDVSHEDPEVKFNWYVDGVEVHNAKTKPREEQYNSTYRVVSVLTVLHQDWLNGKEYKCKVSNKALPAPIEKTISKAKGQPREPQVYTLPPSRDELTKNQVSLTCLVKGFYPSDIAVEWESNGQPENNYKTTPPVLDSDGSFFLYSKLTVDKSRWQQGNVFSCSVMHEALHNHYTQKSLSLSPG

SEQ ID NO: 12 - protein, 339 aa, Artificial Sequence
  Synthetic SARS-CoV-2-RBD-hIgG-Fc Fusion Protein
VIAWNSNNLDSKVGGNYNYLYRLFRKSNLKPFERDISTEIYQAGSTPCNGVEGFNCYFPLQSYGFQPTNGVGYQPYRVVVLSFELLHAPATVGGGGGQGGGGQGGGGQGGGGGDKTHTCPPCPAPELLGGPSVFLFPPKPKDTLMISRTPEVTCVVVDVSHEDPEVKFNWYVDGVEVHNAKTKPREEQYNSTYRVVSVLTVLHQDWLNGKEYKCKVSNKALPAPIEKTISKAKGQPREPQVYTLPPSRDELTKNQVSLTCLVKGFYPSDIAVEWESNGQPENNYKTTPPVLDSDGSFFLYSKLTVDKSRWQQGNVFSCSVMHEALHNHYTQKSLSLSPG

SEQ ID NO: 13 - protein, 273 aa, Artificial Sequence
  Synthetic SARS-Cov-2 RBD Analog
RVQPTESIVRFPNITNLCPFGEVFNATRFASVYAWNRKRISNCVADYSVLYNSASFSTFKCYGVSPTKLNDLCFTNVYADSFVIRGDEVRQIAPGQTGKIADYNYKLPDDFTGCVIAWNSNNLDSKVGGNYNYLYRLFRKSNLKPFERDISTEIYQAGSTPCNGVEGFNCYFPLQSYGFQPTNGVGYQPYRVVVLSFELLHAPATVCGPKKSTNLVKNKCVNFNFNGLTGTGVLTESNKKFLPFQQFGRDIADTTDAVRDPQTLEILDITPCS

SEQ ID NO: 14 - protein, 223 aa, Artificial Sequence
  Synthetic SARS-Cov-2 RBD Analog
RVQPTESIVRFPNITNLCPFGEVFNATRFASVYAWNRKRISNCVADYSVLYNSASFSTFKCYGVSPTKLNDLCFTNVYADSFVIRGDEVRQIAPGQTGKIADYNYKLPDDFTGCVIAWNSNNLDSKVGGNYNYLYRLFRKSNLKPFERDISTEIYQAGSTPCNGVEGFNCYFPLQSYGFQPTNGVGYQPYRVVVLSFELLHAPATVCGPKKSTNLVKNKCVNF

SEQ ID NO: 15 - protein, 217 aa, Artificial Sequence
  Synthetic SARS-Cov-2 RBD Analog
RVQPTESIVRFPNITNLCPFGEVFNATRFASVYAWNRKRISNCVADYSVLYNSASFSTFKCYGVSPTKLNDLCFTNVYADSFVIRGDEVRQIAPGQTGKIADYNYKLPDDFTGCVIAWNSNNLDSKVGGNYNYLYRLFRKSNLKPFERDISTEIYQAGSTPCNGVEGFNCYFPLQSYGFQPTNGVGYQPYRVVVLSFELLHAPATVCGPKKSTNLVK

SEQ ID NO: 16 - protein, 461 aa, Artificial Sequence
  Synthetic SARS-CoV-2-RBD-hIgG-Fc Fusion Protein
RVQPTESIVRFPNITNLCPFGEVFNATRFASVYAWNRKRISNCVADYSVLYNSASFSTFKCYGVSPTKLNDLCFTNVYADSFVIRGDEVRQIAPGQTGKIADYNYKLPDDFTGCVIAWNSNNLDSKVGGNYNYLYRLFRKSNLKPFERDISTEIYQAGSTPCNGVEGFNCYFPLQSYGFQPTNGVGYQPYRVVVLSFELLHAPATVCGPKKSTNLVKNKCVNFGGGSGGGSPKSSDKTHTCPPCPAPELLGGPSVFLFPPKPKDTLMISRTPEVTCVVVDVSHEDPEVKFNWYVDGVEVHNAKTKPREEQYNSTYRVVSVLTVLHQDWLNGKEYKCKVSNKALPAPIEKTISKAKGQPREPQVYTLPPSRDELTKNQVSLTCLVKGFYPSDIAVEWESNGQPENNYKTTPPVLDSDGSFFLYSKLTVDKSRWQQGNVFSCSVMHEALHNHYTQKSLSLSPG

SEQ ID NO: 17 - protein, 462 aa, Artificial Sequence
  Synthetic SARS-CoV-2-RBD-hIgG-Fc Fusion Protein
RVQPTESIVRFPNITNLCPFGEVFNATRFASVYAWNRKRISNCVADYSVLYNSASFSTFKCYGVSPTKLNDLCFTNVYADSFVIRGDEVRQIAPGQTGKIADYNYKLPDDFTGCVIAWNSNNLDSKVGGNYNYLYRLFRKSNLKPFERDISTEIYQAGSTPCNGVEGFNCYFPLQSYGFQPTNGVGYQPYRVVVLSFELLHAPATVCGPKKSTNLVKNKCVNFGGGSGGGSPKSSDKTHTCPPCPAPELLGGPSVFLFPPKPKDTLMISRTPEVTCVVVDVSHEDPEVKFNWYVDGVEVHNAKTKPREEQYNSTYRVVSVLTVLHQDWLNGKEYKCKVSNKALPAPIEKTISKAKGQPREPQVYTLPPSRDELTKNQVSLTCLVKGFYPSDIAVEWESNGQPENNYKTTPPVLDSDGSFFLYSKLTVDKSRWQQGNVFSCSVMHEALHNHYTQKSLSLSPGK

SEQ ID NO: 18 - protein, 470 aa, Artificial Sequence
  Synthetic SARS-CoV-2-RBD-hIgG-Fc Fusion Protein
RVQPTESIVRFPNITNLCPFGEVFNATRFASVYAWNRKRISNCVADYSVLYNSASFSTFKCYGVSPTKLNDLCFTNVYADSFVIRGDEVRQIAPGQTGKIADYNYKLPDDFTGCVIAWNSNNLDSKVGGNYNYLYRLFRKSNLKPFERDISTEIYQAGSTPCNGVEGFNCYFPLQSYGFQPTNGVGYQPYRVVVLSFELLHAPATVCGPKKSTNLVKNKCVNFGGGGGQGGGGQGGGGQGGGGGDKTHTCPPCPAPELLGGPSVFLFPPKPKDTLMISRTPEVTCVVVDVSHEDPEVKFNWYVDGVEVHNAKTKPREEQYNSTYRVVSVLTVLHQDWLNGKEYKCKVSNKALPAPIEKTISKAKGQPREPQVYTLPPSRDELTKNQVSLTCLVKGFYPSDIAVEWESNGQPENNYKTTPPVLDSDGSFFLYSKLTVDKSRWQQGNVFSCSVMHEALHNHYTQKSLSLSPG

SEQ ID NO: 19 - protein, 507 aa, Artificial Sequence
  Synthetic SARS-CoV-2-RBD-hIgG-Fc Fusion Protein
RVQPTESIVRFPNITNLCPFGEVFNATRFASVYAWNRKRISNCVADYSVLYNSASFSTFKCYGVSPTKLNDLCFTNVYADSFVIRGDEVRQIAPGQTGKIADYNYKLPDDFTGCVIAWNSNNLDSKVGGNYNYLYRLFRKSNLKPFERDISTEIYQAGSTPCNGVEGFNCYFPLQSYGFQPTNGVGYQPYRVVVLSFELLHAPATVCGPKKSTNLVKNKCVNFNFNGLTGTGVLTESNKKFLPFQQFGRDIADTTDAVRDPQTLEILDITPCSGGGSGGGSDKTHTCPPCPAPELLGGPSVFLFPPKPKDTLMISRTPEVTCVVVDVSHEDPEVKFNWYVDGVEVHNAKTKPREEQYNSTYRVVSVLTVLHQDWLNGKEYKCKVSNKALPAPIEKTISKAKGQPREPQVYTLPPSRDELTKNQVSLTCLVKGFYPSDIAVEWESNGQPENNYKTTPPVLDSDGSFFLYSKLTVDKSRWQQGNVFSCSVMHEALHNHYTQKSLSLSPG

SEQ ID NO: 20 - protein, 451 aa, Artificial Sequence
  Synthetic SARS-CoV-2-RBD-hIgG-Fc Fusion Protein
RVQPTESIVRFPNITNLCPFGEVFNATRFASVYAWNRKRISNCVADYSVLYNSASFSTFKCYGVSPTKLNDLCFTNVYADSFVIRGDEVRQIAPGQTGKIADYNYKLPDDFTGCVIAWNSNNLDSKVGGNYNYLYRLFRKSNLKPFERDISTEIYQAGSTPCNGVEGFNCYFPLQSYGFQPTNGVGYQPYRVVVLSFELLHAPATVCGPKKSTNLVKGGGSGGGSDKTHTCPPCPAPELLGGPSVFLFPPKPKDTLMISRTPEVTCVVVDVSHEDPEVKFNWYVDGVEVHNAKTKPREEQYNSTYRVVSVLTVLHQDWLNGKEYKCKVSNKALPAPIEKTISKAKGQPREPQVYTLPPSRDELTKNQVSLTCLVKGFYPSDIAVEWESNGQPENNYKTTPPVLDSDGSFFLYSKLTVDKSRWQQGNVFSCSVMHEALHNHYTQKSLSLSPG

SEQ ID NO: 21 - protein, 443 aa, Artificial Sequence
  Synthetic SARS-CoV-2-RBD-hIgG-Fc Fusion Protein
RVQPTESIVRFPNITNLCPFGEVFNATRFASVYAWNRKRISNCVADYSVLYNSASFSTFKCYGVSPTKLNDLCFTNVYADSFVIRGDEVRQIAPGQTGKIADYNYKLPDDFTGCVIAWNSNNLDSKVGGNYNYLYRLFRKSNLKPFERDISTEIYQAGSTPCNGVEGFNCYFPLQSYGFQPTNGVGYQPYRVVVLSFELLHAPATVCGPKKSTNLVKDKTHTCPPCPAPELLGGPSVFLFPPKPKDTLMISRTPEVTCVVVDVSHEDPEVKFNWYVDGVEVHNAKTKPREEQYNSTYRVVSVLTVLHQDWLNGKEYKCKVSNKALPAPIEKTISKAKGQPREPQVYTLPPSRDELTKNQVSLTCLVKGFYPSDIAVEWESNGQPENNYKTTPPVLDSDGSFFLYSKLTVDKSRWQQGNVFSCSVMHEALHNHYTQKSLSLSPG

SEQ ID NO: 22 - protein, 233 aa, Mouse IgG2a Fc Fragment
EPRGPTIKPCPPCKCPAPNLLGGPSVFIFPPKIKDVLMISLSPIVTCVVVDVSEDDPDVQISWFVNNVEVHTAQTQTHREDYNSTLRVVSALPIQHQDWMSGKEFKCKVNNKDLPAPIERTISKPKGSVRAPQVYVLPPPEEEMTKKQVTLTCMVTDFMPEDIYVEWTNNGKTELNYKNTEPVLDSDGSYFMYSKLRVEKKNWVERNSYSCSVVHEGLHNHHTTKSFSRTPGK

SEQ ID NO: 23 - protein, 464 aa, Artificial Sequence
  Synthetic SARS-CoV-2-RBD-Mouse-IgG2a-Fc Fusion Protein
RVQPTESIVRFPNITNLCPFGEVFNATRFASVYAWNRKRISNCVADYSVLYNSASFSTFKCYGVSPTKLNDLCFTNVYADSFVIRGDEVRQIAPGQTGKIADYNYKLPDDFTGCVIAWNSNNLDSKVGGNYNYLYRLFRKSNLKPFERDISTEIYQAGSTPCNGVEGFNCYFPLQSYGFQPTNGVGYQPYRVVVLSFELLHAPATVCGPKKSTNLVKNKCVNFGGGSGGGSEPRGPTIKPCPPCKCPAPNLLGGPSVFIFPPKIKDVLMISLSPIVTCVVVDVSEDDPDVQISWFVNNVEVHTAQTQTHREDYNSTLRVVSALPIQHQDWMSGKEFKCKVNNKDLPAPIERTISKPKGSVRAPQVYVLPPPEEEMTKKQVTLTCMVTDFMPEDIYVEWTNNGKTELNYKNTEPVLDSDGSYFMYSKLRVEKKNWVERNSYSCSVVHEGLHNHHTTKSFSRTPGK

SEQ ID NO: 24 - protein, 254 aa, SARS-Cov-2 RBD UK Variant (N501Y)
PNITNLCPFGEVFNATRFASVYAWNRKRISNCVADYSVLYNSASFSTFKCYGVSPTKLNDLCFTNVYADSFVIRGDEVRQIAPGQTGKIADYNYKLPDDFTGCVIAWNSNNLDSKVGGNYNYLYRLFRKSNLKPFERDISTEIYQAGSTPCNGVEGFNCYFPLQSYGFQPTYGVGYQPYRVVVLSFELLHAPATVCGPKKSTNLVKNKCVNFNFNGLTGTGVLTESNKKFLPFQQFGRDIADTTDAVRDPQTLE

SEQ ID NO: 25 - protein, 254 aa, SARS-Cov-2 RBD South Africa Variant (E484K)
PNITNLCPFGEVFNATRFASVYAWNRKRISNCVADYSVLYNSASFSTFKCYGVSPTKLNDLCFTNVYADSFVIRGDEVRQIAPGQTGKIADYNYKLPDDFTGCVIAWNSNNLDSKVGGNYNYLYRLFRKSNLKPFERDISTEIYQAGSTPCNGVKGFNCYFPLQSYGFQPTNGVGYQPYRVVVLSFELLHAPATVCGPKKSTNLVKNKCVNFNFNGLTGTGVLTESNKKFLPFQQFGRDIADTTDAVRDPQTLE

SEQ ID NO: 26 - protein, 224 aa, Canine Native IgGB
DCPKCPAPEMLGGPSVFIFPPKPKDTLLIARTPEVTCVVVDLDPEDPEVQISWFVDGKQMQTAKTQPREEQFNGTYRVVSVLPIGHQDWLKGKQFTCKVNNKALPSPIERTISKARGQAHQPSVYVLPPSREELSKNTVSLTCLIKDFFPPDIDVEWQSNGQQEPESKYRTTPPQLDEDGSYFLYSKLSVDKSRWQRGDTFICAVMHEALHNHYTQESLSHSPG

SEQ ID NO: 27 - protein, 21 aa, Artificial Sequence
  Synthetic Linker
GGGGGQGGGGQGGGGQGGGGG

SEQ ID NO: 28 - protein, 57 aa, Artificial Sequence
  Synthetic Insulin Analog (B-C-A)
FVNQHLCGSHLVEALELVCGERGFHYGGGGGGSGGGGGIVEQCCTSTCSLDQLENYC

SEQ ID NO: 29 - protein, 302 aa, Artificial Sequence
  Synthetic Canine Insulin-Fc Fusion Protein
FVNQHLCGSHLVEALELVCGERGFHYGGGGGGSGGGGGIVEQCCTSTCSLDQLENYCGGGGGQGGGGQGGGGQGGGGGDCPKCPAPEMLGGPSVFIFPPKPKDTLLIARTPEVTCVVVDLDPEDPEVQISWFVDGKQMQTAKTQPREEQFNGTYRVVSVLPIGHQDWLKGKQFTCKVNNKALPSPIERTISKARGQAHQPSVYVLPPSREELSKNTVSLTCLIKDFFPPDIDVEWQSNGQQEPESKYRTTPPQLDEDGSYFLYSKLSVDKSRWQRGDTFICAVMHEALHNHYTQESLSHSPG

SEQ ID NO: 30 - protein, 224 aa, Artificial Sequence
  Synthetic Fc Fragment
  MISC_FEATURE (73)..(73): Xaa = S, Q, D, K, A
DCPKCPAPEMLGGPSVFIFPPKPKDTLLIARTPEVTCVVVDLDPEDPEVQISWFVDGKQMQTAKTQPREEQFXGTYRVVSVLPIGHQDWLKGKQFTCKVNNKALPSPIERTISKARGQAHQPSVYVLPPSREELSKNTVSLTCLIKDFFPPDIDVEWQSNGQQEPESKYRTTPPQLDEDGSYFLYSKLSVDKSRWQRGDTFICAVMHEALHNHYTQESLSHSPG

SEQ ID NO: 31 - protein, 57 aa, Artificial Sequence
  Synthetic Insulin Analog (B-C-A)
FVNQHLCGSHLVEALALVCGERGFHYGGGGGGSGGGGGIVEQCCTSTCSLDQLENYC

SEQ ID NO: 32 - protein, 302 aa, Artificial Sequence
  Synthetic Canine Insulin-Fc Fusion Protein
FVNQHLCGSHLVEALALVCGERGFHYGGGGGGSGGGGGIVEQCCTSTCSLDQLENYCGGGGGQGGGGQGGGGQGGGGGDCPKCPAPEMLGGPSVFIFPPKPKDTLLIARTPEVTCVVVDLDPEDPEVQISWFVDGKQMQTAKTQPREEQFSGTYRVVSVLPIGHQDWLKGKQFTCKVNNKALPSPIERTISKARGQAHQPSVYVLPPSREELSKNTVSLTCLIKDFFPPDIDVEWQSNGQQEPESKYRTTPPQLDEDGSYFLYSKLSVDKSRWQRGDTFICAVMHEALHNHYTQESLSHSPG

SEQ ID NO: 33 - protein, 230 aa, Artificial Sequence
  Synthetic Fc Fragment
PKSSDKTHTCPPCPAPELLGGPSVFLFPPKPKDTLMISRTPEVTCVVVDVSHEDPEVKFNWYVDGVEVHNAKTKPREEQYNSTYRVVSVLTVLHQDWLNGKEYKCKVSNKALPAPIEKTISKAKGQPREPQVYTLPPSRDELTKNQVSLTCLVKGFYPSDIAVEWESNGQPENNYKTTPPVLDSDGSFFLYSKLTVDKSRWQQGNVFSCSVMHEALHNHYTQKSLSLSPG